European Patent Application EP 4 306 165 A2, published January 17, 2024. Title: COMPOSITIONS, USES AND METHODS FOR TREATMENT OF METABOLIC DISORDERS AND DISEASES. Applicant: NGM Biopharmaceuticals, Inc. The sequence listing filed with the application follows.

SEQUENCE LISTING (168 sequences)

SEQ ID NO: 1 - protein, 194 aa, Homo sapiens
RPLAFSDASPHVHYGWGDPIRLRHLYTSGPHGLSSCFLRIRADGVVDCARGQSAHSLLEIKAVALRTVAIKGVHSVRYLCMGADGKMQGLLQYSEEDCAFEEEIRPDGYNVYRSEKHRLPVSLSSAKQRQLYKNRGFLPLSHFLPMLPMVPEEPEDLRGHLESDMFSSPLETDSMDPFGLVTGLEAVRSPSFEK

SEQ ID NO: 2 - protein, 194 aa, Homo sapiens
RPLAFSDSSPLVHYGWGDPIRLRHLYTSGPHGLSSCFLRIRADGVVDCARGQSAHSLLEIKAVALRTVAIKGVHSVRYLCMGADGKMQGLLQYSEEDCAFEEEIRPDGYNVYRSEKHRLPVSLSSAKQRQLYKNRGFLPLSHFLPMLPMVPEEPEDLRGHLESDMFSSPLETDSMDPFGLVTGLEAVRSPSFEK

SEQ ID NO: 3 - protein, 194 aa, Homo sapiens
RPLAFSDAGPHVHYGWGDPIRLRHLYTSGPHGLSSCFLRIRADGVVDCARGQSAHSLLEIKAVALRTVAIKGVHSVRYLCMGADGKMQGLLQYSEEDCAFEEEILEDGYNVYRSEKHRLPVSLSSAKQRQLYKNRGFLPLSHFLPMLPMVPEEPEDLRGHLESDMFSSPLETDSMDPFGLVTGLEAVRSPSFEK

SEQ ID NO: 4 - protein, 194 aa, Homo sapiens
RPLAFSDAGPHVHYAWGDPIRLRHLYTSGPHGLSSCFLRIRADGVVDCARGQSAHSLLEIKAVALRTVAIKGVHSVRYLCMGADGKMQGLLQYSEEDCAFEEEIRPDGYNVYRSEKHRLPVSLSSAKQRQLYKNRGFLPLSHFLPMLPMVPEEPEDLRGHLESDMFSSPLETDSMDPFGLVTGLEAVRSPSFEK

SEQ ID NO: 5 - protein, 191 aa, Homo sapiens
RHPIPDSSPLLQFGGQVRLRHLYTSGPHGLSSCFLRIRADGVVDCARGQSAHSLLEIKAVALRTVAIKGVHSVRYLCMGADGKMQGLLQYSEEDCAFEEEIRPDGYNVYRSEKHRLPVSLSSAKQRQLYKNRGFLPLSHFLPMLPMVPEEPEDLRGHLESDMFSSPLETDSMDPFGLVTGLEAVRSPSFEK

SEQ ID NO: 6 - protein, 187 aa, Homo sapiens
RDSSPLLQFGGQVRLRHLYTSGPHGLSSCFLRIRADGVVDCARGQSAHSLLEIKAVALRTVAIKGVHSVRYLCMGADGKMQGLLQYSEEDCAFEEEIRPDGYNVYRSEKHRLPVSLSSAKQRQLYKNRGFLPLSHFLPMLPMVPEEPEDLRGHLESDMFSSPLETDSMDPFGLVTGLEAVRSPSFEK

SEQ ID NO: 7 - protein, 192 aa, Homo sapiens
RPLAFSDSSPLLQFGGQVRLRHLYTSGPHGLSSCFLRIRADGVVDCARGQSAHSLLEIKAVALRTVAIKGVHSVRYLCMGADGKMQGLLQYSEEDCAFEEEIRPDGYNVYRSEKHRLPVSLSSAKQRQLYKNRGFLPLSHFLPMLPMVPEEPEDLRGHLESDMFSSPLETDSMDPFGLVTGLEAVRSPSFEK

SEQ ID NO: 8 - protein, 191 aa, Homo sapiens
RHPIPDSSPLLQWGDPIRLRHLYTSGPHGLSSCFLRIRADGVVDCARGQSAHSLLEIKAVALRTVAIKGVHSVRYLCMGADGKMQGLLQYSEEDCAFEEEIRPDGYNVYRSEKHRLPVSLSSAKQRQLYKNRGFLPLSHFLPMLPMVPEEPEDLRGHLESDMFSSPLETDSMDPFGLVTGLEAVRSPSFEK

SEQ ID NO: 9 - protein, 193 aa, Homo sapiens
RHPIPDSSPLLQFGWGDPIRLRHLYTSGPHGLSSCFLRIRADGVVDCARGQSAHSLLEIKAVALRTVAIKGVHSVRYLCMGADGKMQGLLQYSEEDCAFEEEIRPDGYNVYRSEKHRLPVSLSSAKQRQLYKNRGFLPLSHFLPMLPMVPEEPEDLRGHLESDMFSSPLETDSMDPFGLVTGLEAVRSPSFEK

SEQ ID NO: 10 - protein, 193 aa, Homo sapiens
RHPIPDSSPHVHYGWGDPIRLRHLYTSGPHGLSSCFLRIRADGVVDCARGQSAHSLLEIKAVALRTVAIKGVHSVRYLCMGADGKMQGLLQYSEEDCAFEEEIRPDGYNVYRSEKHRLPVSLSSAKQRQLYKNRGFLPLSHFLPMLPMVPEEPEDLRGHLESDMFSSPLETDSMDPFGLVTGLEAVRSPSFEK

SEQ ID NO: 11 - protein, 192 aa, Homo sapiens
RPLAFSDAGPLLQWGDPIRLRHLYTSGPHGLSSCFLRIRADGVVDCARGQSAHSLLEIKAVALRTVAIKGVHSVRYLCMGADGKMQGLLQYSEEDCAFEEEIRPDGYNVYRSEKHRLPVSLSSAKQRQLYKNRGFLPLSHFLPMLPMVPEEPEDLRGHLESDMFSSPLETDSMDPFGLVTGLEAVRSPSFEK

SEQ ID NO: 12 - protein, 194 aa, Homo sapiens
RPLAFSDAGPLLQFGWGDPIRLRHLYTSGPHGLSSCFLRIRADGVVDCARGQSAHSLLEIKAVALRTVAIKGVHSVRYLCMGADGKMQGLLQYSEEDCAFEEEIRPDGYNVYRSEKHRLPVSLSSAKQRQLYKNRGFLPLSHFLPMLPMVPEEPEDLRGHLESDMFSSPLETDSMDPFGLVTGLEAVRSPSFEK

SEQ ID NO: 13 - protein, 192 aa, Homo sapiens
RPLAFSDAGPLLQFGGQVRLRHLYTSGPHGLSSCFLRIRADGVVDCARGQSAHSLLEIKAVALRTVAIKGVHSVRYLCMGADGKMQGLLQYSEEDCAFEEEIRPDGYNVYRSEKHRLPVSLSSAKQRQLYKNRGFLPLSHFLPMLPMVPEEPEDLRGHLESDMFSSPLETDSMDPFGLVTGLEAVRSPSFEK

SEQ ID NO: 14 - protein, 191 aa, Homo sapiens
RHPIPDSSPHVHYGGQVRLRHLYTSGPHGLSSCFLRIRADGVVDCARGQSAHSLLEIKAVALRTVAIKGVHSVRYLCMGADGKMQGLLQYSEEDCAFEEEIRPDGYNVYRSEKHRLPVSLSSAKQRQLYKNRGFLPLSHFLPMLPMVPEEPEDLRGHLESDMFSSPLETDSMDPFGLVTGLEAVRSPSFEK

SEQ ID NO: 15 - protein, 192 aa, Homo sapiens
RPLAFSDAGPHVHWGDPIRLRHLYTSGPHGLSSCFLRIRADGVVDCARGQSAHSLLEIKAVALRTVAIKGVHSVRYLCMGADGKMQGLLQYSEEDCAFEEEIRPDGYNVYRSEKHRLPVSLSSAKQRQLYKNRGFLPLSHFLPMLPMVPEEPEDLRGHLESDMFSSPLETDSMDPFGLVTGLEAVRSPSFEK

SEQ ID NO: 16 - protein, 192 aa, Homo sapiens; identical to SEQ ID NO: 15

SEQ ID NO: 17 - protein, 192 aa, Homo sapiens
RPLAFSDAGPHVGWGDPIRLRHLYTSGPHGLSSCFLRIRADGVVDCARGQSAHSLLEIKAVALRTVAIKGVHSVRYLCMGADGKMQGLLQYSEEDCAFEEEIRPDGYNVYRSEKHRLPVSLSSAKQRQLYKNRGFLPLSHFLPMLPMVPEEPEDLRGHLESDMFSSPLETDSMDPFGLVTGLEAVRSPSFEK

SEQ ID NO: 18 - protein, 192 aa, Homo sapiens
RPLAFSDAGPHYGWGDPIRLRHLYTSGPHGLSSCFLRIRADGVVDCARGQSAHSLLEIKAVALRTVAIKGVHSVRYLCMGADGKMQGLLQYSEEDCAFEEEIRPDGYNVYRSEKHRLPVSLSSAKQRQLYKNRGFLPLSHFLPMLPMVPEEPEDLRGHLESDMFSSPLETDSMDPFGLVTGLEAVRSPSFEK

SEQ ID NO: 19 - protein, 192 aa, Homo sapiens
RPLAFSDAGPVYGWGDPIRLRHLYTSGPHGLSSCFLRIRADGVVDCARGQSAHSLLEIKAVALRTVAIKGVHSVRYLCMGADGKMQGLLQYSEEDCAFEEEIRPDGYNVYRSEKHRLPVSLSSAKQRQLYKNRGFLPLSHFLPMLPMVPEEPEDLRGHLESDMFSSPLETDSMDPFGLVTGLEAVRSPSFEK

SEQ ID NO: 20 - protein, 192 aa, Homo sapiens
RPLAFSDAGPVHGWGDPIRLRHLYTSGPHGLSSCFLRIRADGVVDCARGQSAHSLLEIKAVALRTVAIKGVHSVRYLCMGADGKMQGLLQYSEEDCAFEEEIRPDGYNVYRSEKHRLPVSLSSAKQRQLYKNRGFLPLSHFLPMLPMVPEEPEDLRGHLESDMFSSPLETDSMDPFGLVTGLEAVRSPSFEK

SEQ ID NO: 21 - protein, 192 aa, Homo sapiens
RPLAFSDAGPVHYWGDPIRLRHLYTSGPHGLSSCFLRIRADGVVDCARGQSAHSLLEIKAVALRTVAIKGVHSVRYLCMGADGKMQGLLQYSEEDCAFEEEIRPDGYNVYRSEKHRLPVSLSSAKQRQLYKNRGFLPLSHFLPMLPMVPEEPEDLRGHLESDMFSSPLETDSMDPFGLVTGLEAVRSPSFEK

SEQ ID NO: 22 - protein, 193 aa, Homo sapiens
RPLAFSDAGPHVHGWGDPIRLRHLYTSGPHGLSSCFLRIRADGVVDCARGQSAHSLLEIKAVALRTVAIKGVHSVRYLCMGADGKMQGLLQYSEEDCAFEEEIRPDGYNVYRSEKHRLPVSLSSAKQRQLYKNRGFLPLSHFLPMLPMVPEEPEDLRGHLESDMFSSPLETDSMDPFGLVTGLEAVRSPSFEK

SEQ ID NO: 23 - protein, 192 aa, Homo sapiens
RPLAFSDAGPHHGWGDPIRLRHLYTSGPHGLSSCFLRIRADGVVDCARGQSAHSLLEIKAVALRTVAIKGVHSVRYLCMGADGKMQGLLQYSEEDCAFEEEIRPDGYNVYRSEKHRLPVSLSSAKQRQLYKNRGFLPLSHFLPMLPMVPEEPEDLRGHLESDMFSSPLETDSMDPFGLVTGLEAVRSPSFEK

SEQ ID NO: 24 - protein, 192 aa, Homo sapiens
RPLAFSDAGPHHYWGDPIRLRHLYTSGPHGLSSCFLRIRADGVVDCARGQSAHSLLEIKAVALRTVAIKGVHSVRYLCMGADGKMQGLLQYSEEDCAFEEEIRPDGYNVYRSEKHRLPVSLSSAKQRQLYKNRGFLPLSHFLPMLPMVPEEPEDLRGHLESDMFSSPLETDSMDPFGLVTGLEAVRSPSFEK

SEQ ID NO: 25 - protein, 192 aa, Homo sapiens
RPLAFSDAGPHVYWGDPIRLRHLYTSGPHGLSSCFLRIRADGVVDCARGQSAHSLLEIKAVALRTVAIKGVHSVRYLCMGADGKMQGLLQYSEEDCAFEEEIRPDGYNVYRSEKHRLPVSLSSAKQRQLYKNRGFLPLSHFLPMLPMVPEEPEDLRGHLESDMFSSPLETDSMDPFGLVTGLEAVRSPSFEK

SEQ ID NO: 26 - protein, 192 aa, Homo sapiens
RPLAFSDSSPLVHWGDPIRLRHLYTSGPHGLSSCFLRIRADGVVDCARGQSAHSLLEIKAVALRTVAIKGVHSVRYLCMGADGKMQGLLQYSEEDCAFEEEIRPDGYNVYRSEKHRLPVSLSSAKQRQLYKNRGFLPLSHFLPMLPMVPEEPEDLRGHLESDMFSSPLETDSMDPFGLVTGLEAVRSPSFEK

SEQ ID NO: 27 - protein, 192 aa, Homo sapiens
RPLAFSDSSPHVHWGDPIRLRHLYTSGPHGLSSCFLRIRADGVVDCARGQSAHSLLEIKAVALRTVAIKGVHSVRYLCMGADGKMQGLLQYSEEDCAFEEEIRPDGYNVYRSEKHRLPVSLSSAKQRQLYKNRGFLPLSHFLPMLPMVPEEPEDLRGHLESDMFSSPLETDSMDPFGLVTGLEAVRSPSFEK

SEQ ID NO: 28 - protein, 191 aa, Homo sapiens
RPLAFSDAGPHVWGDPIRLRHLYTSGPHGLSSCFLRIRADGVVDCARGQSAHSLLEIKAVALRTVAIKGVHSVRYLCMGADGKMQGLLQYSEEDCAFEEEIRPDGYNVYRSEKHRLPVSLSSAKQRQLYKNRGFLPLSHFLPMLPMVPEEPEDLRGHLESDMFSSPLETDSMDPFGLVTGLEAVRSPSFEK

SEQ ID NO: 29 - protein, 193 aa, Homo sapiens
RPLAFSDAGPHVHYWGDPIRLRHLYTSGPHGLSSCFLRIRADGVVDCARGQSAHSLLEIKAVALRTVAIKGVHSVRYLCMGADGKMQGLLQYSEEDCAFEEEIRPDGYNVYRSEKHRLPVSLSSAKQRQLYKNRGFLPLSHFLPMLPMVPEEPEDLRGHLESDMFSSPLETDSMDPFGLVTGLEAVRSPSFEK

SEQ ID NO: 30 - protein, 194 aa, Homo sapiens; identical to SEQ ID NO: 4

SEQ ID NO: 31 - protein, 191 aa, Homo sapiens
RHPIPDSSPLLQFGAQVRLRHLYTSGPHGLSSCFLRIRADGVVDCARGQSAHSLLEIKAVALRTVAIKGVHSVRYLCMGADGKMQGLLQYSEEDCAFEEEIRPDGYNVYRSEKHRLPVSLSSAKQRQLYKNRGFLPLSHFLPMLPMVPEEPEDLRGHLESDMFSSPLETDSMDPFGLVTGLEAVRSPSFEK

SEQ ID NO: 32 - protein, 191 aa, Homo sapiens
RHPIPDSSPLLQFGDQVRLRHLYTSGPHGLSSCFLRIRADGVVDCARGQSAHSLLEIKAVALRTVAIKGVHSVRYLCMGADGKMQGLLQYSEEDCAFEEEIRPDGYNVYRSEKHRLPVSLSSAKQRQLYKNRGFLPLSHFLPMLPMVPEEPEDLRGHLESDMFSSPLETDSMDPFGLVTGLEAVRSPSFEK

SEQ ID NO: 33 - protein, 191 aa, Homo sapiens
RHPIPDSSPLLQFGPQVRLRHLYTSGPHGLSSCFLRIRADGVVDCARGQSAHSLLEIKAVALRTVAIKGVHSVRYLCMGADGKMQGLLQYSEEDCAFEEEIRPDGYNVYRSEKHRLPVSLSSAKQRQLYKNRGFLPLSHFLPMLPMVPEEPEDLRGHLESDMFSSPLETDSMDPFGLVTGLEAVRSPSFEK

SEQ ID NO: 34 - protein, 191 aa, Homo sapiens
RHPIPDSSPLLQFGGAVRLRHLYTSGPHGLSSCFLRIRADGVVDCARGQSAHSLLEIKAVALRTVAIKGVHSVRYLCMGADGKMQGLLQYSEEDCAFEEEIRPDGYNVYRSEKHRLPVSLSSAKQRQLYKNRGFLPLSHFLPMLPMVPEEPEDLRGHLESDMFSSPLETDSMDPFGLVTGLEAVRSPSFEK

SEQ ID NO: 35 - protein, 191 aa, Homo sapiens
RHPIPDSSPLLQFGGEVRLRHLYTSGPHGLSSCFLRIRADGVVDCARGQSAHSLLEIKAVALRTVAIKGVHSVRYLCMGADGKMQGLLQYSEEDCAFEEEIRPDGYNVYRSEKHRLPVSLSSAKQRQLYKNRGFLPLSHFLPMLPMVPEEPEDLRGHLESDMFSSPLETDSMDPFGLVTGLEAVRSPSFEK

SEQ ID NO: 36 - protein, 191 aa, Homo sapiens
RHPIPDSSPLLQFGGNVRLRHLYTSGPHGLSSCFLRIRADGVVDCARGQSAHSLLEIKAVALRTVAIKGVHSVRYLCMGADGKMQGLLQYSEEDCAFEEEIRPDGYNVYRSEKHRLPVSLSSAKQRQLYKNRGFLPLSHFLPMLPMVPEEPEDLRGHLESDMFSSPLETDSMDPFGLVTGLEAVRSPSFEK

SEQ ID NO: 37 - protein, 191 aa, Homo sapiens
RHPIPDSSPLLQFGGQARLRHLYTSGPHGLSSCFLRIRADGVVDCARGQSAHSLLEIKAVALRTVAIKGVHSVRYLCMGADGKMQGLLQYSEEDCAFEEEIRPDGYNVYRSEKHRLPVSLSSAKQRQLYKNRGFLPLSHFLPMLPMVPEEPEDLRGHLESDMFSSPLETDSMDPFGLVTGLEAVRSPSFEK

SEQ ID NO: 38 - protein, 191 aa, Homo sapiens
RHPIPDSSPLLQFGGQIRLRHLYTSGPHGLSSCFLRIRADGVVDCARGQSAHSLLEIKAVALRTVAIKGVHSVRYLCMGADGKMQGLLQYSEEDCAFEEEIRPDGYNVYRSEKHRLPVSLSSAKQRQLYKNRGFLPLSHFLPMLPMVPEEPEDLRGHLESDMFSSPLETDSMDPFGLVTGLEAVRSPSFEK

SEQ ID NO: 39 - protein, 191 aa, Homo sapiens
RHPIPDSSPLLQFGGQTRLRHLYTSGPHGLSSCFLRIRADGVVDCARGQSAHSLLEIKAVALRTVAIKGVHSVRYLCMGADGKMQGLLQYSEEDCAFEEEIRPDGYNVYRSEKHRLPVSLSSAKQRQLYKNRGFLPLSHFLPMLPMVPEEPEDLRGHLESDMFSSPLETDSMDPFGLVTGLEAVRSPSFEK

SEQ ID NO: 40 - protein, 193 aa, Homo sapiens
RHPIPDSSPLLQFGWGQPVRLRHLYTSGPHGLSSCFLRIRADGVVDCARGQSAHSLLEIKAVALRTVAIKGVHSVRYLCMGADGKMQGLLQYSEEDCAFEEEIRPDGYNVYRSEKHRLPVSLSSAKQRQLYKNRGFLPLSHFLPMLPMVPEEPEDLRGHLESDMFSSPLETDSMDPFGLVTGLEAVRSPSFEK

SEQ ID NO: 41 - protein, 182 aa, Homo sapiens
RPLAFSDAGPHVHYGWGDPIRLRHLYTSGPHGLSSCFLRIRADGVVDCARGQSAHSLLEIKAVALRTVAIKGVHSVRYLCMGADGKMQGLLQYSEEDCAFEEEIRPDGYNVYRSEKHRLPVSLSSAKQRQLYKNRGFLPLSHFLPMLPEPPGILAPQPPDVGSSDPLSMVGPSQGRSPSYAS

SEQ ID NO: 42 - protein, 178 aa, Homo sapiens
HPIPDSSPLLQFGGQVRLRHLYTSGPHGLSSCFLRIRADGVVDCARGQSAHSLLEIKAVALRTVAIKGVHSVRYLCMGADGKMQGLLQYSEEDCAFEEEIRPDGYNVYRSEKHRLPVSLSSAKQRQLYKNRGFLPLSHFLPMLPEPPGILAPQPPDVGSSDPLSMVGPSQGRSPSYAS

SEQ ID NO: 43 - protein, 192 aa, Homo sapiens
RPLAFSDAGPHVHYGGDIRLRHLYTSGPHGLSSCFLRIRADGVVDCARGQSAHSLLEIKAVALRTVAIKGVHSVRYLCMGADGKMQGLLQYSEEDCAFEEEIRPDGYNVYRSEKHRLPVSLSSAKQRQLYKNRGFLPLSHFLPMLPMVPEEPEDLRGHLESDMFSSPLETDSMDPFGLVTGLEAVRSPSFEK

SEQ ID NO: 44 - protein, 185 aa, Homo sapiens
RPLAFSDAGPHVHYGWGDPIRQRYLYTDDAQQTEAHLEIREDGTVGGAADQSPESLLQLKALKPGVIQILGVKTSRFLCQRPDGALYGSLHFDPEACSFRELLLEDGYNVYQSEAHGLPLHLPGNKSPHRDPAPRGPARFLPLPGLPPALPEPPGILAPQPPDVGSSDPLSMVGPSQGRSPSYAS

SEQ ID NO: 45 - protein, 193 aa, Homo sapiens
HPIPDSSPLLQFGGQVRQRYLYTDDAQQTEAHLEIREDGTVGGAADQSPESLLQLKALKPGVIQILGVKTSRFLCQRPDGALYGSLHFDPEACSFRELLLEDGYNVYQSEAHGLPLHLPGNKSPHRDPAPRGPARFLPLPGLPPALPMVPEEPEDLRGHLESDMFSSPLETDSMDPFGLVTGLEAVRSPSFEK

SEQ ID NO: 46 - protein, 232 aa, Homo sapiens
RPLAFSDAGPHVHYGWGDPIRQRYLYTDDAQQTEAHLEIREDGTVGGAADQSPESLLQLKALKPGVIQILGVKTSRFLCQRPDGALYGSLHFDPEACSFRELLLEDGYNVYQSEAHGLPLHLPGNKSPHRDPAPRGPARFLPLPGLPPALPEPPGILAPQPPDVGSSDPLSMVGPSQGRSPSYASPMVPEEPEDLRGHLESDMFSSPLETDSMDPFGLVTGLEAVRSPSFEK

SEQ ID NO: 47 - protein, 190 aa, Homo sapiens
HPIPDSSPLLQWGDPIRLRHLYTSGPHGLSSCFLRIRADGVVDCARGQSAHSLLEIKAVALRTVAIKGVHSVRYLCMGADGKMQGLLQYSEEDCAFEEEIRPDGYNVYRSEKHRLPVSLSSAKQRQLYKNRGFLPLSHFLPMLPMVPEEPEDLRGHLESDMFSSPLETDSMDPFGLVTGLEAVRSPSFEK

SEQ ID NO: 48 - protein, 187 aa, Homo sapiens; identical to SEQ ID NO: 6

SEQ ID NO: 49 - protein, 192 aa, Homo sapiens; identical to SEQ ID NO: 7

SEQ ID NO: 50 - protein, 191 aa, Homo sapiens
RHPIPDSSPLLQFGDQVRLRHLYTSGPHGLSSCFLRIRADGVVDCARGQSAHSLLEIKAVALRTVAIKGVHSVRYLCMGADGKMQGLLQYSEEDCAFEEEILEDGYNVYRSEKHRLPVSLSSAKQRQLYKNRGFLPLSHFLPMLPMVPEEPEDLRGHLESDMFSSPLETDSMDPFGLVTGLEAVRSPSFEK

SEQ ID NO: 51 - protein, 191 aa, Homo sapiens; identical to SEQ ID NO: 36

SEQ ID NO: 52 - protein, 187 aa, Homo sapiens
RDSSPLLQWGDPIRLRHLYTSGPHGLSSCFLRIRADGVVDCARGQSAHSLLEIKAVALRTVAIKGVHSVRYLCMGADGKMQGLLQYSEEDCAFEEEIRPDGYNVYRSEKHRLPVSLSSAKQRQLYKNRGFLPLSHFLPMLPMVPEEPEDLRGHLESDMFSSPLETDSMDPFGLVTGLEAVRSPSFEK

SEQ ID NO: 53 - protein, 189 aa, Homo sapiens
MDSSPLVHYGWGDPIRLRHLYTSGPHGLSSCFLRIRADGVVDCARGQSAHSLLEIKAVALRTVAIKGVHSVRYLCMGADGKMQGLLQYSEEDCAFEEEIRPDGYNVYRSEKHRLPVSLSSAKQRQLYKNRGFLPLSHFLPMLPMVPEEPEDLRGHLESDMFSSPLETDSMDPFGLVTGLEAVRSPSFEK

SEQ ID NO: 54 - protein, 192 aa, Homo sapiens; identical to SEQ ID NO: 11

SEQ ID NO: 55 - protein, 192 aa, Homo sapiens; identical to SEQ ID NO: 18

SEQ ID NO: 56 - protein, 192 aa, Homo sapiens; identical to SEQ ID NO: 19

SEQ ID NO: 57 - protein, 192 aa, Homo sapiens; identical to SEQ ID NO: 20

SEQ ID NO: 58 - protein, 192 aa, Homo sapiens; identical to SEQ ID NO: 21

SEQ ID NO: 59 - protein, 192 aa, Homo sapiens; identical to SEQ ID NO: 23

SEQ ID NO: 60 - protein, 192 aa, Homo sapiens; identical to SEQ ID NO: 24

SEQ ID NO: 61 - protein, 192 aa, Homo sapiens; identical to SEQ ID NO: 17

SEQ ID NO: 62 - protein, 192 aa, Homo sapiens; identical to SEQ ID NO: 25

SEQ ID NO: 63 - protein, 192 aa, Homo sapiens; identical to SEQ ID NO: 15

SEQ ID NO: 64 - protein, 192 aa, Homo sapiens; identical to SEQ ID NO: 26

SEQ ID NO: 65 - protein, 192 aa, Homo sapiens; identical to SEQ ID NO: 27

SEQ ID NO: 66 - protein, 192 aa, Homo sapiens
RPLAFSDAGPHLQWGDPIRLRHLYTSGPHGLSSCFLRIRADGVVDCARGQSAHSLLEIKAVALRTVAIKGVHSVRYLCMGADGKMQGLLQYSEEDCAFEEEIRPDGYNVYRSEKHRLPVSLSSAKQRQLYKNRGFLPLSHFLPMLPMVPEEPEDLRGHLESDMFSSPLETDSMDPFGLVTGLEAVRSPSFEK

SEQ ID NO: 67 - protein, 191 aa, Homo sapiens; identical to SEQ ID NO: 28

SEQ ID NO: 68 - protein, 193 aa, Homo sapiens; identical to SEQ ID NO: 29

SEQ ID NO: 69 - protein, 189 aa, Homo sapiens
RDSSPLVHYGWGDPIRLRHLYTSGPHGLSSCFLRIRADGVVDCARGQSAHSLLEIKAVALRTVAIKGVHSVRYLCMGADGKMQGLLQYSEEDCAFEEEIRPDGYNVYRSEKHRLPVSLSSAKQRQLYKNRGFLPLSHFLPMLPMVPEEPEDLRGHLESDMFSSPLETDSMDPFGLVTGLEAVRSPSFEK

SEQ ID NO: 70 - protein, 190 aa, Homo sapiens
MRDSSPLVHYGWGDPIRLRHLYTSGPHGLSSCFLRIRADGVVDCARGQSAHSLLEIKAVALRTVAIKGVHSVRYLCMGADGKMQGLLQYSEEDCAFEEEIRPDGYNVYRSEKHRLPVSLSSAKQRQLYKNRGFLPLSHFLPMLPMVPEEPEDLRGHLESDMFSSPLETDSMDPFGLVTGLEAVRSPSFEK

SEQ ID NO: 71 - protein, 181 aa, Homo sapiens
HPIPDSSPLLQFGGQVRQRYLYTDDAQQTEAHLEIREDGTVGGAADQSPESLLQLKALKPGVIQILGVKTSRFLCQRPDGALYGSLHFDPEACSFRELLLEDGYNVYQSEAHSLPLHLPGNKSPHRDPAPRGPARFLPLPGLPPALPEPPGILAPQPPDVGSSDPLSMVGPSQGRSPSYAS

SEQ ID NO: 72 - protein, 181 aa, Homo sapiens
HPIPDSSPLLQFGGQVRQRYLYTDDAQQTEAHLEIREDGTVGGAADQSPESLLQLKALKPGVIQILGVKTSRFLCQRPDGALYGSLHFDPEACSFRELLLEDGYNVYQSEAHGLPLHLPGNKSPHRDPAPRGPARFLPLPGLPPAPPEPPGILAPQPPDVGSSDPLSMVGPSQGRSPSYAS

SEQ ID NO: 73 - protein, 212 aa, Homo sapiens
HPIPDSSPLLQFGGQVRQRYLYTDDAQQTEAHLEIREDGTVGGAADQSPESLLQLKALKPGVIQILGVKTSRFLCQRPDGALYGSLHFDPEACSFRELLLEDGYNVYQSEAHGLPLHLPGNKSPHRDPAPRGPARFLPLPGLPPALPEPPGILAPQPPDVGSSDPLSMVVQDELQGVGGEGCHMHPENCKTLLTDIDRTHTEKPVWDGITGE

SEQ ID NO: 74 - protein, 189 aa, Homo sapiens
RDAGPHVHYGWGDPIRLRHLYTSGPHGLSSCFLRIRADGVVDCARGQSAHSLLEIKAVALRTVAIKGVHSVRYLCMGADGKMQGLLQYSEEDCAFEEEIRPDGYNVYRSEKHRLPVSLSSAKQRQLYKNRGFLPLSHFLPMLPMVPEEPEDLRGHLESDMFSSPLETDSMDPFGLVTGLEAVRSPSFEK

SEQ ID NO: 75 - protein, 184 aa, Homo sapiens
RVHYGWGDPIRLRHLYTSGPHGLSSCFLRIRADGVVDCARGQSAHSLLEIKAVALRTVAIKGVHSVRYLCMGADGKMQGLLQYSEEDCAFEEEIRPDGYNVYRSEKHRLPVSLSSAKQRQLYKNRGFLPLSHFLPMLPMVPEEPEDLRGHLESDMFSSPLETDSMDPFGLVTGLEAVRSPSFEK

SEQ ID NO: 76 - protein, 179 aa, Homo sapiens
RGDPIRLRHLYTSGPHGLSSCFLRIRADGVVDCARGQSAHSLLEIKAVALRTVAIKGVHSVRYLCMGADGKMQGLLQYSEEDCAFEEEIRPDGYNVYRSEKHRLPVSLSSAKQRQLYKNRGFLPLSHFLPMLPMVPEEPEDLRGHLESDMFSSPLETDSMDPFGLVTGLEAVRSPSFEK

SEQ ID NO: 77 - protein, 175 aa, Homo sapiens
RRLRHLYTSGPHGLSSCFLRIRADGVVDCARGQSAHSLLEIKAVALRTVAIKGVHSVRYLCMGADGKMQGLLQYSEEDCAFEEEIRPDGYNVYRSEKHRLPVSLSSAKQRQLYKNRGFLPLSHFLPMLPMVPEEPEDLRGHLESDMFSSPLETDSMDPFGLVTGLEAVRSPSFEK

SEQ ID NO: 78 - protein, 188 aa, Homo sapiens
RAGPHVHYGWGDPIRLRHLYTSGPHGLSSCFLRIRADGVVDCARGQSAHSLLEIKAVALRTVAIKGVHSVRYLCMGADGKMQGLLQYSEEDCAFEEEIRPDGYNVYRSEKHRLPVSLSSAKQRQLYKNRGFLPLSHFLPMLPMVPEEPEDLRGHLESDMFSSPLETDSMDPFGLVTGLEAVRSPSFEK

SEQ ID NO: 79 - protein, 187 aa, Homo sapiens
RGPHVHYGWGDPIRLRHLYTSGPHGLSSCFLRIRADGVVDCARGQSAHSLLEIKAVALRTVAIKGVHSVRYLCMGADGKMQGLLQYSEEDCAFEEEIRPDGYNVYRSEKHRLPVSLSSAKQRQLYKNRGFLPLSHFLPMLPMVPEEPEDLRGHLESDMFSSPLETDSMDPFGLVTGLEAVRSPSFEK

SEQ ID NO: 80 - protein, 186 aa, Homo sapiens
RPHVHYGWGDPIRLRHLYTSGPHGLSSCFLRIRADGVVDCARGQSAHSLLEIKAVALRTVAIKGVHSVRYLCMGADGKMQGLLQYSEEDCAFEEEIRPDGYNVYRSEKHRLPVSLSSAKQRQLYKNRGFLPLSHFLPMLPMVPEEPEDLRGHLESDMFSSPLETDSMDPFGLVTGLEAVRSPSFEK

SEQ ID NO: 81 - protein, 185 aa, Homo sapiens
RHVHYGWGDPIRLRHLYTSGPHGLSSCFLRIRADGVVDCARGQSAHSLLEIKAVALRTVAIKGVHSVRYLCMGADGKMQGLLQYSEEDCAFEEEIRPDGYNVYRSEKHRLPVSLSSAKQRQLYKNRGFLPLSHFLPMLPMVPEEPEDLRGHLESDMFSSPLETDSMDPFGLVTGLEAVRSPSFEK

SEQ ID NO: 82 - protein, 194 aa, Homo sapiens
RPLAFSAAGPHVHYGWGDPIRLRHLYTSGPHGLSSCFLRIRADGVVDCARGQSAHSLLEIKAVALRTVAIKGVHSVRYLCMGADGKMQGLLQYSEEDCAFEEEIRPDGYNVYRSEKHRLPVSLSSAKQRQLYKNRGFLPLSHFLPMLPMVPEEPEDLRGHLESDMFSSPLETDSMDPFGLVTGLEAVRSPSFEK

SEQ ID NO: 83 - protein, 194 aa, Homo sapiens
RPLAFSDAAPHVHYGWGDPIRLRHLYTSGPHGLSSCFLRIRADGVVDCARGQSAHSLLEIKAVALRTVAIKGVHSVRYLCMGADGKMQGLLQYSEEDCAFEEEIRPDGYNVYRSEKHRLPVSLSSAKQRQLYKNRGFLPLSHFLPMLPMVPEEPEDLRGHLESDMFSSPLETDSMDPFGLVTGLEAVRSPSFEK

SEQ ID NO: 84 - protein, 194 aa, Homo sapiens
RPLAFSDAGAHVHYGWGDPIRLRHLYTSGPHGLSSCFLRIRADGVVDCARGQSAHSLLEIKAVALRTVAIKGVHSVRYLCMGADGKMQGLLQYSEEDCAFEEEIRPDGYNVYRSEKHRLPVSLSSAKQRQLYKNRGFLPLSHFLPMLPMVPEEPEDLRGHLESDMFSSPLETDSMDPFGLVTGLEAVRSPSFEK

SEQ ID NO: 85 - protein, 194 aa, Homo sapiens
RPLAFSDAGPHVHYGAGDPIRLRHLYTSGPHGLSSCFLRIRADGVVDCARGQSAHSLLEIKAVALRTVAIKGVHSVRYLCMGADGKMQGLLQYSEEDCAFEEEIRPDGYNVYRSEKHRLPVSLSSAKQRQLYKNRGFLPLSHFLPMLPMVPEEPEDLRGHLESDMFSSPLETDSMDPFGLVTGLEAVRSPSFEK

SEQ ID NO: 86 - protein, 194 aa, Homo sapiens
RPLAFSDAGPHVHYGWGAPIRLRHLYTSGPHGLSSCFLRIRADGVVDCARGQSAHSLLEIKAVALRTVAIKGVHSVRYLCMGADGKMQGLLQYSEEDCAFEEEIRPDGYNVYRSEKHRLPVSLSSAKQRQLYKNRGFLPLSHFLPMLPMVPEEPEDLRGHLESDMFSSPLETDSMDPFGLVTGLEAVRSPSFEK

SEQ ID NO: 87 - protein, 167 aa, Homo sapiens
RPLAFSDAGPHVHYGWGDAICARGQSAHSLLEIKAVALRTVAIKGVHSVRYLCMGADGKMQGLLQYSEEDCAFEEEIRPDGYNVYRSEKHRLPVSLSSAKQRQLYKNRGFLPLSHFLPMLPMVPEEPEDLRGHLESDMFSSPLETDSMDPFGLVTGLEAVRSPSFEK

SEQ ID NO: 88 - protein, 194 aa, Homo sapiens
RPLAFSDAGPHVHYGWGDPIRLRHLYTSGPAGLSSCFLRIRADGVVDCARGQSAHSLLEIKAVALRTVAIKGVHSVRYLCMGADGKMQGLLQYSEEDCAFEEEIRPDGYNVYRSEKHRLPVSLSSAKQRQLYKNRGFLPLAHFLPMLPMVPEEPEDLRGHLESDMFSSPLETDSMDPFGLVTGLEAVRSPSFEK

SEQ ID NO: 89 - protein, 194 aa, Homo sapiens
RPLAFSDAGPHVHYGWGDPIRLRHLYTSGPAGLSSCFLRIRADGVVDCARGQSAHSLLEIKAVALRTVAIKGVHSVRYLCMGADGKMQGLLQYSEEDCAFEEEIRPDGYNVYRSEKHRLPVSLSSAKQRQLYKNRGFLPLSAFLPMLPMVPEEPEDLRGHLESDMFSSPLETDSMDPFGLVTGLEAVRSPSFEK

SEQ ID NO: 90 - protein, 194 aa, Homo sapiens
RPLAFSDAGPHVHYGWGDPIRLRHLYTSGPHGLSSCFLRIRADGVVDCARGQSAHSLLEIKAVALRTVAIKGVHSVRYLCMGADGKMQGLLQYSEEDCAFEEEIRPDGYNVYRSEKHRLPVSLSSAAQAQLYKNRGFLPLSHFLPMLPMVPEEPEDLRGHLESDMFSSPLETDSMDPFGLVTGLEAVRSPSFEK

SEQ ID NO: 91 - protein, 194 aa, Homo sapiens
RPLAFSDAGPHVHYGWGDPIRLRHLYTSGPHGLSSCFLRIRADGVVDCARGQSAHSLLEIKAVALRTVAIKGVHSVRYLCMGADGKMQGLLQYSEEDCAFEEEIRPDGYNVYRSEKHRLPVSLSSAAQRQLYKNRGFLPLAHFLPMLPMVPEEPEDLRGHLESDMFSSPLETDSMDPFGLVTGLEAVRSPSFEK

SEQ ID NO: 92 - protein, 194 aa, Homo sapiens
RPLAFSDAGPHVHYGWGDPIRLRHLYTSGPHGLSSCFLRIRADGVVDCARGQSAHSLLEIKAVALRTVAIKGVHSVRYLCMGADGKMQGLLQYSEEDCAFEEEIRPDGYNVYRSEKHRLPVSLSSAAQRQLYKNRGFLPLSAFLPMLPMVPEEPEDLRGHLESDMFSSPLETDSMDPFGLVTGLEAVRSPSFEK

SEQ ID NO: 93 - protein, 194 aa, Homo sapiens
RPLAFSDAGPHVHYGWGDPIRLRHLYTSGPHGLSSCFLRIRADGVVDCARGQSAHSLLEIKAVALRTVAIKGVHSVRYLCMGADGKMQGLLQYSEEDCAFEEEIRPDGYNVYRSEKHRLPVSLSSAKQAQLYKNRGFLPLAHFLPMLPMVPEEPEDLRGHLESDMFSSPLETDSMDPFGLVTGLEAVRSPSFEK

SEQ ID NO: 94 - protein, 194 aa, Homo sapiens
RPLAFSDAGPHVHYGWGDPIRLRHLYTSGPHGLSSCFLRIRADGVVDCARGQSAHSLLEIKAVALRTVAIKGVHSVRYLCMGADGKMQGLLQYSEEDCAFEEEIRPDGYNVYRSEKHRLPVSLSSAKQRQLYKNRGFLPLAAFLPMLPMVPEEPEDLRGHLESDMFSSPLETDSMDPFGLVTGLEAVRSPSFEK

SEQ ID NO: 95 - protein, 194 aa, Homo sapiens; identical to SEQ ID NO: 92

SEQ ID NO: 96 - protein, 194 aa, Homo sapiens
RPLAFSDAGPHVHYGWGDPIRLRHLYTSGPHGLSSCFLRIRADGVVDCARGQSAHSLLEIKAVALRTVAIKGVHSVRYLCMGADGKMQGLLQYSEEDCAFEEEIRPDGYNVYRSEKHRLPVSLSSAAQAQLYKNRGFLPLAHFLPMLPMVPEEPEDLRGHLESDMFSSPLETDSMDPFGLVTGLEAVRSPSFEK

SEQ ID NO: 97 - protein, 194 aa, Homo sapiens
RPLAFSDAGPHVHYGWGDPIRLRHLYTSGPHGLSSCFLRIRADGVVDCARGQSAHSLLEIKAVALRTVAIKGVHSVRYLCMGADGKMQGLLQYSEEDCAFEEEIRPDGYNVYRSEKHRLPVSLSSAAQAQLYKNRGFLPLSAFLPMLPMVPEEPEDLRGHLESDMFSSPLETDSMDPFGLVTGLEAVRSPSFEK

SEQ ID NO: 98 - protein, 194 aa, Homo sapiens
RPLAFSDAGPHVHYGWGDPIRLRHLYTSGPHGLSSCFLRIRADGVVDCARGQSAHSLLEIKAVALRTVAIKGVHSVRYLCMGADGKMQGLLQYSEEDCAFEEEIRPDGYNVYRSEKHRLPVSLSSAAQAQLYKNRGFLPLAAFLPMLPMVPEEPEDLRGHLESDMFSSPLETDSMDPFGLVTGLEAVRSPSFEK

SEQ ID NO: 99 - protein, 194 aa, Homo sapiens
RPLAFSDAGPHVHYGWGDPIRLRHLYTSGPHGLSSCFLRIRADGVVDCARGQSAHSLLEIKAVALRTVAIKGVHSVRYLCMGADGKMQGLLQYSEEDCAFEEEIRPDGYNVYRSEKHRLPVSLSSAKQRQLYKNRGFLPLSHFLPMLPMVPEEPEDLRGHLESDMFSSPLETDSMDPFGLVTGLEAVRSPSFEK

SEQ ID NO: 100 - protein, 181 aa, Homo sapiens
HPIPDSSPLLQFGGQVRQRYLYTDDAQQTEAHLEIREDGTVGGAADQSPESLLQLKALKPGVIQILGVKTSRFLCQRPDGALYGSLHFDPEACSFRELLLEDGYNVYQSEAHGLPLHLPGNKSPHRDPAPRGPARFLPLPGLPPALPEPPGILAPQPPDVGSSDPLSMVGPSQGRSPSYAS

SEQ ID NO: 101 - protein, 4 aa, Homo sapiens
VHYG

SEQ ID NO: 102 - protein, 9 aa, Homo sapiens
DASPHVHYG

SEQ ID NO: 103 - protein, 9 aa, Homo sapiens
DSSPLVHYG

SEQ ID NO: 104 - protein, 7 aa, Homo sapiens
DSSPLLQ

SEQ ID NO: 105 - protein, 12 aa, Homo sapiens
DSSPLLQFGGQV

SEQ ID NO: 106 - protein, 5 aa, Homo sapiens
RHPIP

SEQ ID NO: 107 - protein, 4 aa, Homo sapiens
HPIP

SEQ ID NO: 108 - protein, 5 aa, Homo sapiens
RPLAF

SEQ ID NO: 109 - protein, 4 aa, Homo sapiens
PLAF

SEQ ID NO: 110 - protein, 6 aa, Homo sapiens
MDSSPL

SEQ ID NO: 111 - protein, 7 aa, Homo sapiens
MSDSSPL

SEQ ID NO: 112 - protein, 6 aa, Homo sapiens
SDSSPL

SEQ ID NO: 113 - protein, 5 aa, Homo sapiens
MSSPL

SEQ ID NO: 114 - protein, 4 aa, Homo sapiens
SSPL

SEQ ID NO: 115 - protein, 4 aa, Homo sapiens
RDSS

SEQ ID NO: 116 - protein, 4 aa, Homo sapiens
MDSS

SEQ ID NO: 117 - protein, 5 aa, Homo sapiens
MRDSS

SEQ ID NO: 118 - protein, 5 aa, Homo sapiens
MSSPL

SEQ ID NO: 119 - protein, 6 aa, Homo sapiens
MDSSPL

SEQ ID NO: 120 - protein, 7 aa, Homo sapiens
MSDSSPL

SEQ ID NO: 121 - protein, 5 aa, Homo sapiens
DSSPL

SEQ ID NO: 122 - protein, 5 aa, Homo sapiens
DASPH

SEQ ID NO: 123 - protein, 4 aa, Homo sapiens
RDSS

SEQ ID NO: 124 - protein, 4 aa, Homo sapiens
MDSS

SEQ ID NO: 125 - protein, 5 aa, Homo sapiens
MRDSS

SEQ ID NO: 126 - protein, 6 aa, Homo sapiens
MDSSPL

SEQ ID NO: 127 - protein, 7 aa, Homo sapiens
MSDSSPL

SEQ ID NO: 128 - protein, 5 aa, Homo sapiens
MSSPL

SEQ ID NO: 129 - protein, 5 aa, synthetic construct
  source 1..5: note = Linker sequence
GSGGS

SEQ ID NO: 130 - protein, 4 aa, synthetic construct
  source 1..4: note = Linker sequence
GGGS

SEQ ID NO: 131 - protein, 4 aa, synthetic construct
  source 1..4: note = Linker sequence
GGSG

SEQ ID NO: 132 - protein, 5 aa, synthetic construct
  source 1..5: note = Linker sequence
GGSGG

SEQ ID NO: 133 - protein, 5 aa, synthetic construct
  source 1..5: note = Linker sequence
GSGSG

SEQ ID NO: 134 - protein, 5 aa, synthetic construct
  source 1..5: note = Linker sequence
GSGGG

SEQ ID NO: 135 - protein, 5 aa, synthetic construct
  source 1..5: note = Linker sequence
GSSSG

SEQ ID NO: 136 - DNA, 32 bp, synthetic construct
  source 1..32: mol_type = other DNA; note = Forward primer
ccgactagtcaccatgcggagcgggtgtgtgg

SEQ ID NO: 137 - DNA, 41 bp, synthetic construct
  source 1..41: mol_type = other DNA; note = Reverse primer
ataagaatgcggccgcttacttctcaaagctgggactcctc

SEQ ID NO: 138 - protein, 186 aa, Homo sapiens
DSSPLLQFGGQVRLRHLYTSGPHGLSSCFLRIRADGVVDCARGQSAHSLLEIKAVALRTVAIKGVHSVRYLCMGADGKMQGLLQYSEEDCAFEEEIRPDGYNVYRSEKHRLPVSLSSAKQRQLYKNRGFLPLSHFLPMLPMVPEEPEDLRGHLESDMFSSPLETDSMDPFGLVTGLEAVRSPSFEK

SEQ ID NO: 139 - protein, 194 aa, Homo sapiens; identical to SEQ ID NO: 1

SEQ ID NO: 140 - protein, 194 aa, Homo sapiens; identical to SEQ ID NO: 2

SEQ ID NO: 141 - protein, 188 aa, Homo sapiens
DSSPLVHYGWGDPIRLRHLYTSGPHGLSSCFLRIRADGVVDCARGQSAHSLLEIKAVALRTVAIKGVHSVRYLCMGADGKMQGLLQYSEEDCAFEEEIRPDGYNVYRSEKHRLPVSLSSAKQRQLYKNRGFLPLSHFLPMLPMVPEEPEDLRGHLESDMFSSPLETDSMDPFGLVTGLEAVRSPSFEK

SEQ ID NO: 142 - protein, 193 aa, Homo sapiens; identical to SEQ ID NO: 9

SEQ ID NO: 143 - protein, 191 aa, Homo sapiens; identical to SEQ ID NO: 8

SEQ ID NO: 144 - protein, 194 aa, Homo sapiens; identical to SEQ ID NO: 12

SEQ ID NO: 145 - protein, 193 aa, Homo sapiens; identical to SEQ ID NO: 10

SEQ ID NO: 146 - protein, 192 aa, Homo sapiens; identical to SEQ ID NO: 13

SEQ ID NO: 147 - protein, 191 aa, Homo sapiens; identical to SEQ ID NO: 14

SEQ ID NO: 148 - protein, 187 aa, Homo sapiens; identical to SEQ ID NO: 6

SEQ ID NO: 149 - protein, 192 aa, Homo sapiens; identical to SEQ ID NO: 7

SEQ ID NO: 150 - protein, 191 aa, Homo sapiens; identical to SEQ ID NO: 31

SEQ ID NO: 151 - protein, 191 aa, Homo sapiens; identical to SEQ ID NO: 32

SEQ ID NO: 152 - protein, 191 aa, Homo sapiens; identical to SEQ ID NO: 33

SEQ ID NO: 153 - protein, 191 aa, Homo sapiens; identical to SEQ ID NO: 34

SEQ ID NO: 154 - protein, 191 aa, Homo sapiens; identical to SEQ ID NO: 35

SEQ ID NO: 155 - protein, 191 aa, Homo sapiens; identical to SEQ ID NO: 36

SEQ ID NO: 156 - protein, 191 aa, Homo sapiens; identical to SEQ ID NO: 37

SEQ ID NO: 157 - protein, 191 aa, Homo sapiens; identical to SEQ ID NO: 38

SEQ ID NO: 158 - protein, 191 aa, Homo sapiens; identical to SEQ ID NO: 39

SEQ ID NO: 159 - protein, 193 aa, Homo sapiens; identical to SEQ ID NO: 40

SEQ ID NO: 160 - protein, 190 aa, Homo sapiens
HPIPDSSPLLQFGGQVRLRHLYTSGPHGLSSCFLRIRADGVVDCARGQSAHSLLEIKAVALRTVAIKGVHSVRYLCMGADGKMQGLLQYSEEDCAFEEEIRPDGYNVYRSEKHRLPVSLSSAKQRQLYKNRGFLPLSHFLPMLPMVPEEPEDLRGHLESDMFSSPLETDSMDPFGLVTGLEAVRSPSFEK

SEQ ID NO: 161 - protein, 186 aa, Homo sapiens; identical to SEQ ID NO: 138

SEQ ID NO: 162 - protein, 190 aa, Homo sapiens; identical to SEQ ID NO: 47

SEQ ID NO: 163 - protein, 192 aa, Homo sapiens
HPIPDSSPLLQFGWGDPIRLRHLYTSGPHGLSSCFLRIRADGVVDCARGQSAHSLLEIKAVALRTVAIKGVHSVRYLCMGADGKMQGLLQYSEEDCAFEEEIRPDGYNVYRSEKHRLPVSLSSAKQRQLYKNRGFLPLSHFLPMLPMVPEEPEDLRGHLESDMFSSPLETDSMDPFGLVTGLEAVRSPSFEK

SEQ ID NO: 164 - protein, 192 aa, Homo sapiens
HPIPDSSPHVHYGWGDPIRLRHLYTSGPHGLSSCFLRIRADGVVDCARGQSAHSLLEIKAVALRTVAIKGVHSVRYLCMGADGKMQGLLQYSEEDCAFEEEIRPDGYNVYRSEKHRLPVSLSSAKQRQLYKNRGFLPLSHFLPMLPMVPEEPEDLRGHLESDMFSSPLETDSMDPFGLVTGLEAVRSPSFEK

SEQ ID NO: 165 - protein, 190 aa, Homo sapiens
HPIPDSSPHVHYGGQVRLRHLYTSGPHGLSSCFLRIRADGVVDCARGQSAHSLLEIKAVALRTVAIKGVHSVRYLCMGADGKMQGLLQYSEEDCAFEEEIRPDGYNVYRSEKHRLPVSLSSAKQRQLYKNRGFLPLSHFLPMLPMVPEEPEDLRGHLESDMFSSPLETDSMDPFGLVTGLEAVRSPSFEK

SEQ ID NO: 166 - protein, 188 aa, Homo sapiens
DAGPHVHYGWGDPIRLRHLYTSGPHGLSSCFLRIRADGVVDCARGQSAHSLLEIKAVALRTVAIKGVHSVRYLCMGADGKMQGLLQYSEEDCAFEEEIRPDGYNVYRSEKHRLPVSLSSAKQRQLYKNRGFLPLSHFLPMLPMVPEEPEDLRGHLESDMFSSPLETDSMDPFGLVTGLEAVRSPSFEK

SEQ ID NO: 167 - protein, 183 aa, Homo sapiens
VHYGWGDPIRLRHLYTSGPHGLSSCFLRIRADGVVDCARGQSAHSLLEIKAVALRTVAIKGVHSVRYLCMGADGKMQGLLQYSEEDCAFEEEIRPDGYNVYRSEKHRLPVSLSSAKQRQLYKNRGFLPLSHFLPMLPMVPEEPEDLRGHLESDMFSSPLETDSMDPFGLVTGLEAVRSPSFEK

SEQ ID NO: 168 - protein, 174 aa, Homo sapiens
RLRHLYTSGPHGLSSCFLRIRADGVVDCARGQSAHSLLEIKAVALRTVAIKGVHSVRYLCMGADGKMQGLLQYSEEDCAFEEEIRPDGYNVYRSEKHRLPVSLSSAKQRQLYKNRGFLPLSHFLPMLPMVPEEPEDLRGHLESDMFSSPLETDSMDPFGLVTGLEAVRSPSFEK